European Patent Specification EP 4 149 511 B1, published March 25, 2026. Title: MITOCHONDRIAL-DERIVED PEPTIDES AND ANALOGS THEREOF FOR USE AS A THERAPY FOR AGE-RELATED DISEASES INCLUDING CANCER. Applicant: UNIVERSITY OF SOUTHERN CALIFORNIA COHEN, Pinchas YEN, Kelvin KIM, Su-Jeong. The sequence listing filed with the application follows.

SEQUENCE LISTING (215 sequences)

SEQ ID NO: 1 - protein, 32 aa, Artificial Sequence
  synthetic construct
MRLFGLLLAVRRDGRSLSLMLTLIRGLSKRLG

SEQ ID NO: 2 - protein, 32 aa, Artificial Sequence
  synthetic construct
MRLFGLLLAVRRSGRSLSLMLTLIRGLDKRLG

SEQ ID NO: 3 - protein, 32 aa, Artificial Sequence
  synthetic construct
MRLFGLLLAVRRDGRSLSLMLDLIRGLDKRLG

SEQ ID NO: 4 - protein, 20 aa, Artificial Sequence
  synthetic construct
GLLLAVRRSGRSLDLMLTLI

SEQ ID NO: 5 - protein, 16 aa, Artificial Sequence
  synthetic construct
MRLFGLLLAVRRSGRS

SEQ ID NO: 6 - protein, 16 aa, Artificial Sequence
  synthetic construct
LSLMLTLIRGLSKRLG

SEQ ID NO: 7 - protein, 32 aa, Artificial Sequence
  synthetic construct
MRLFGLLLAVGGSGRSLSLMLTLIRGLSKRLG

SEQ ID NO: 8 - protein, 32 aa, Artificial Sequence
  synthetic construct
MRLFGLLLAVGGSGGSLSLMLTLIRGLSKRLG

SEQ ID NO: 9 - protein, 32 aa, Artificial Sequence
  synthetic construct
  MOD_RES (1)..(1): FORMYLATION
MRLFGLLLAVRRSGRSLSLMLTLIRGLSKRLG

SEQ ID NO: 10 - protein, 32 aa, Artificial Sequence
  synthetic construct
MRLFGLLLAVRRDGRDLDLMLDLIRGLDKRLG

SEQ ID NO: 11 - protein, 32 aa, Artificial Sequence
  synthetic construct
MRLFGLLLAVRRDGRDLDLMLDLIRGLSKRLG

SEQ ID NO: 12 - protein, 32 aa, Artificial Sequence
  synthetic construct
MRLFGLLLAVRRSGRDLDLMLDLIRGLDKRLG

SEQ ID NO: 13 - protein, 32 aa, Artificial Sequence
  synthetic construct
MRLFGLLLAVRRDGRSLDLMLDLIRGLDKRLG

SEQ ID NO: 14 - protein, 32 aa, Artificial Sequence
  synthetic construct
MRLFGLLLAVRRDGRDLSLMLDLIRGLDKRLG

SEQ ID NO: 15 - protein, 32 aa, Artificial Sequence
  synthetic construct
MRLFGLLLAVRRDGRDLDLMLTLIRGLDKRLG

SEQ ID NO: 16 - protein, 32 aa, Artificial Sequence
  synthetic construct
MRLFGLLLAVRRDGRDLDLMLTLIRGLSKRLG

SEQ ID NO: 17 - protein, 32 aa, Artificial Sequence
  synthetic construct
MRLFGLLLAVRRDGRDLSLMLDLIRGLSKRLG

SEQ ID NO: 18 - protein, 32 aa, Artificial Sequence
  synthetic construct
MRLFGLLLAVRRDGRDLSLMLTLIRGLDKRLG

SEQ ID NO: 19 - protein, 32 aa, Artificial Sequence
  synthetic construct
MRLFGLLLAVRRDGRSLDLMLDLIRGLSKRLG

SEQ ID NO: 20 - protein, 32 aa, Artificial Sequence
  synthetic construct
MRLFGLLLAVRRDGRSLDLMLTLIRGLDKRLG

SEQ ID NO: 21 - protein, 32 aa, Artificial Sequence
  synthetic construct
MRLFGLLLAVRRSGRDLDLMLDLIRGLSKRLG

SEQ ID NO: 22 - protein, 32 aa, Artificial Sequence
  synthetic construct
MRLFGLLLAVRRSGRDLDLMLTLIRGLDKRLG

SEQ ID NO: 23 - protein, 32 aa, Artificial Sequence
  synthetic construct
MRLFGLLLAVRRSGRDLSLMLDLIRGLDKRLG

SEQ ID NO: 24 - protein, 32 aa, Artificial Sequence
  synthetic construct
MRLFGLLLAVRRSGRSLDLMLDLIRGLDKRLG

SEQ ID NO: 25 - protein, 32 aa, Artificial Sequence
  synthetic construct
MRLFGLLLAVRRDGRDLSLMLTLIRGLSKRLG

SEQ ID NO: 26 - protein, 32 aa, Artificial Sequence
  synthetic construct
MRLFGLLLAVRRDGRSLDLMLTLIRGLSKRLG

SEQ ID NO: 27 - protein, 32 aa, Artificial Sequence
  synthetic construct
MRLFGLLLAVRRDGRSLSLMLDLIRGLSKRLG

SEQ ID NO: 28 - protein, 32 aa, Artificial Sequence
  synthetic construct
MRLFGLLLAVRRDGRSLSLMLTLIRGLDKRLG

SEQ ID NO: 29 - protein, 32 aa, Artificial Sequence
  synthetic construct
MRLFGLLLAVRRSGRDLDLMLTLIRGLSKRLG

SEQ ID NO: 30 - protein, 32 aa, Artificial Sequence
  synthetic construct
MRLFGLLLAVRRSGRDLSLMLDLIRGLSKRLG

SEQ ID NO: 31 - protein, 32 aa, Artificial Sequence
  synthetic construct
MRLFGLLLAVRRSGRDLSLMLTLIRGLDKRLG

SEQ ID NO: 32 - protein, 32 aa, Artificial Sequence
  synthetic construct
MRLFGLLLAVRRSGRSLDLMLDLIRGLSKRLG

SEQ ID NO: 33 - protein, 32 aa, Artificial Sequence
  synthetic construct
MRLFGLLLAVRRSGRSLDLMLTLIRGLDKRLG

SEQ ID NO: 34 - protein, 32 aa, Artificial Sequence
  synthetic construct
MRLFGLLLAVRRSGRSLSLMLDLIRGLDKRLG

SEQ ID NO: 35 - protein, 32 aa, Artificial Sequence
  synthetic construct
ARLFGLLLAVRRSGRSLSLMLTLIRGLSKRLG

SEQ ID NO: 36 - protein, 32 aa, Artificial Sequence
  synthetic construct
MALFGLLLAVRRSGRSLSLMLTLIRGLSKRLG

SEQ ID NO: 37 - protein, 32 aa, Artificial Sequence
  synthetic construct
MRAFGLLLAVRRSGRSLSLMLTLIRGLSKRLG

SEQ ID NO: 38 - protein, 32 aa, Artificial Sequence
  synthetic construct
MRLAGLLLAVRRSGRSLSLMLTLIRGLSKRLG

SEQ ID NO: 39 - protein, 32 aa, Artificial Sequence
  synthetic construct
MRLFALLLAVRRSGRSLSLMLTLIRGLSKRLG

SEQ ID NO: 40 - protein, 32 aa, Artificial Sequence
  synthetic construct
MRLFGALLAVRRSGRSLSLMLTLIRGLSKRLG

SEQ ID NO: 41 - protein, 32 aa, Artificial Sequence
  synthetic construct
MRLFGLALAVRRSGRSLSLMLTLIRGLSKRLG

SEQ ID NO: 42 - protein, 32 aa, Artificial Sequence
  synthetic construct
MRLFGLLAAVRRSGRSLSLMLTLIRGLSKRLG

SEQ ID NO: 43 - protein, 32 aa, Artificial Sequence
  synthetic construct
MRLFGLLLAARRSGRSLSLMLTLIRGLSKRLG

SEQ ID NO: 44 - protein, 32 aa, Artificial Sequence
  synthetic construct
MRLFGLLLAVARSGRSLSLMLTLIRGLSKRLG

SEQ ID NO: 45 - protein, 32 aa, Artificial Sequence
  synthetic construct
MRLFGLLLAVRASGRSLSLMLTLIRGLSKRLG

SEQ ID NO: 46 - protein, 32 aa, Artificial Sequence
  synthetic construct
MRLFGLLLAVRRAGRSLSLMLTLIRGLSKRLG

SEQ ID NO: 47 - protein, 32 aa, Artificial Sequence
  synthetic construct
MRLFGLLLAVRRSARSLSLMLTLIRGLSKRLG

SEQ ID NO: 48 - protein, 32 aa, Artificial Sequence
  synthetic construct
MRLFGLLLAVRRSGASLSLMLTLIRGLSKRLG

SEQ ID NO: 49 - protein, 32 aa, Artificial Sequence
  synthetic construct
MRLFGLLLAVRRSGRALSLMLTLIRGLSKRLG

SEQ ID NO: 50 - protein, 32 aa, Artificial Sequence
  synthetic construct
MRLFGLLLAVRRSGRSASLMLTLIRGLSKRLG

SEQ ID NO: 51 - protein, 32 aa, Artificial Sequence
  synthetic construct
MRLFGLLLAVRRSGRSLALMLTLIRGLSKRLG

SEQ ID NO: 52 - protein, 32 aa, Artificial Sequence
  synthetic construct
MRLFGLLLAVRRSGRSLSAMLTLIRGLSKRLG

SEQ ID NO: 53 - protein, 32 aa, Artificial Sequence
  synthetic construct
MRLFGLLLAVRRSGRSLSLALTLIRGLSKRLG

SEQ ID NO: 54 - protein, 32 aa, Artificial Sequence
  synthetic construct
MRLFGLLLAVRRSGRSLSLMATLIRGLSKRLG

SEQ ID NO: 55 - protein, 32 aa, Artificial Sequence
  synthetic construct
MRLFGLLLAVRRSGRSLSLMLALIRGLSKRLG

SEQ ID NO: 56 - protein, 32 aa, Artificial Sequence
  synthetic construct
MRLFGLLLAVRRSGRSLSLMLTAIRGLSKRLG

SEQ ID NO: 57 - protein, 32 aa, Artificial Sequence
  synthetic construct
MRLFGLLLAVRRSGRSLSLMLTLARGLSKRLG

SEQ ID NO: 58 - protein, 32 aa, Artificial Sequence
  synthetic construct
MRLFGLLLAVRRSGRSLSLMLTLIAGLSKRLG

SEQ ID NO: 59 - protein, 32 aa, Artificial Sequence
  synthetic construct
MRLFGLLLAVRRSGRSLSLMLTLIRALSKRLG

SEQ ID NO: 60 - protein, 32 aa, Artificial Sequence
  synthetic construct
MRLFGLLLAVRRSGRSLSLMLTLIRGASKRLG

SEQ ID NO: 61 - protein, 32 aa, Artificial Sequence
  synthetic construct
MRLFGLLLAVRRSGRSLSLMLTLIRGLAKRLG

SEQ ID NO: 62 - protein, 32 aa, Artificial Sequence
  synthetic construct
MRLFGLLLAVRRSGRSLSLMLTLIRGLSARLG

SEQ ID NO: 63 - protein, 32 aa, Artificial Sequence
  synthetic construct
MRLFGLLLAVRRSGRSLSLMLTLIRGLSKALG

SEQ ID NO: 64 - protein, 32 aa, Artificial Sequence
  synthetic construct
MRLFGLLLAVRRSGRSLSLMLTLIRGLSKRAG

SEQ ID NO: 65 - protein, 32 aa, Artificial Sequence
  synthetic construct
MRLFGLLLAVRRSGRSLSLMLTLIRGLSKRLA

SEQ ID NO: 66 - protein, 28 aa, Artificial Sequence
  synthetic construct
RLFGLLLAVGGSGGSLSLMLTLIRGLSK

SEQ ID NO: 67 - protein, 24 aa, Artificial Sequence
  synthetic construct
RLFGLLLAVGGLSLMLTLIRGLSK

SEQ ID NO: 68 - protein, 30 aa, Artificial Sequence
  synthetic construct
RLFGLLLAVGGSGGSGGLSLMLTLIRGLSK

SEQ ID NO: 69 - protein, 16 aa, Artificial Sequence
  synthetic construct
MRLFGLLLAVGGSGGS

SEQ ID NO: 70 - protein, 22 aa, Artificial Sequence
  synthetic construct
GGSGGSLSLMLTLIRGLSKRLG

SEQ ID NO: 71 - protein, 17 aa, Artificial Sequence
  synthetic construct
LLAVGGSGGSLSLMLTL

SEQ ID NO: 72 - protein, 24 aa, Artificial Sequence
  synthetic construct
LLLAVGGSGGSLSLMLTLIRGLSK

SEQ ID NO: 73 - protein, 32 aa, Artificial Sequence
  synthetic construct
MRLFGLLLAVPGSGGSLSLMLTLIRGLSKRLG

SEQ ID NO: 74 - protein, 32 aa, Artificial Sequence
  synthetic construct
MRLFGLLLAVPGSGPSLSLMLTLIRGLSKRLG

SEQ ID NO: 75 - protein, 32 aa, Artificial Sequence
  synthetic construct
MRLFGLLLAVRRSGGSLSLMLTLIRGLSKRLG

SEQ ID NO: 76 - protein, 24 aa, Artificial Sequence
  synthetic construct
LLLAVGGSGGDLDLMLTLIRGLDK

SEQ ID NO: 77 - protein, 32 aa, Artificial Sequence
  synthetic construct
MPLFGLLLAVRRSGRSLSLMLTLIRGLSKRLG

SEQ ID NO: 78 - protein, 32 aa, Artificial Sequence
  synthetic construct
MRPFGLLLAVRRSGRSLSLMLTLIRGLSKRLG

SEQ ID NO: 79 - protein, 32 aa, Artificial Sequence
  synthetic construct
MRLPGLLLAVRRSGRSLSLMLTLIRGLSKRLG

SEQ ID NO: 80 - protein, 32 aa, Artificial Sequence
  synthetic construct
MRLFPLLLAVRRSGRSLSLMLTLIRGLSKRLG

SEQ ID NO: 81 - protein, 32 aa, Artificial Sequence
  synthetic construct
MRLFGPLLAVRRSGRSLSLMLTLIRGLSKRLG

SEQ ID NO: 82 - protein, 32 aa, Artificial Sequence
  synthetic construct
MRLFGLPLAVRRSGRSLSLMLTLIRGLSKRLG

SEQ ID NO: 83 - protein, 32 aa, Artificial Sequence
  synthetic construct
MRLFGLLPAVRRSGRSLSLMLTLIRGLSKRLG

SEQ ID NO: 84 - protein, 32 aa, Artificial Sequence
  synthetic construct
MRLFGLLLPVRRSGRSLSLMLTLIRGLSKRLG

SEQ ID NO: 85 - protein, 32 aa, Artificial Sequence
  synthetic construct
MRLFGLLLAPRRSGRSLSLMLTLIRGLSKRLG

SEQ ID NO: 86 - protein, 32 aa, Artificial Sequence
  synthetic construct
MRLFGLLLAVPRSGRSLSLMLTLIRGLSKRLG

SEQ ID NO: 87 - protein, 32 aa, Artificial Sequence
  synthetic construct
MRLFGLLLAVRPSGRSLSLMLTLIRGLSKRLG

SEQ ID NO: 88 - protein, 32 aa, Artificial Sequence
  synthetic construct
MRLFGLLLAVRRPGRSLSLMLTLIRGLSKRLG

SEQ ID NO: 89 - protein, 32 aa, Artificial Sequence
  synthetic construct
MRLFGLLLAVRRSPRSLSLMLTLIRGLSKRLG

SEQ ID NO: 90 - protein, 32 aa, Artificial Sequence
  synthetic construct
MRLFGLLLAVRRSGPSLSLMLTLIRGLSKRLG

SEQ ID NO: 91 - protein, 32 aa, Artificial Sequence
  synthetic construct
MRLFGLLLAVRRSGRPLSLMLTLIRGLSKRLG

SEQ ID NO: 92 - protein, 32 aa, Artificial Sequence
  synthetic construct
MRLFGLLLAVRRSGRSPSLMLTLIRGLSKRLG

SEQ ID NO: 93 - protein, 32 aa, Artificial Sequence
  synthetic construct
MRLFGLLLAVRRSGRSLPLMLTLIRGLSKRLG

SEQ ID NO: 94 - protein, 32 aa, Artificial Sequence
  synthetic construct
MRLFGLLLAVRRSGRSLSPMLTLIRGLSKRLG

SEQ ID NO: 95 - protein, 32 aa, Artificial Sequence
  synthetic construct
MRLFGLLLAVRRSGRSLSLPLTLIRGLSKRLG

SEQ ID NO: 96 - protein, 32 aa, Artificial Sequence
  synthetic construct
MRLFGLLLAVRRSGRSLSLMPTLIRGLSKRLG

SEQ ID NO: 97 - protein, 32 aa, Artificial Sequence
  synthetic construct
MRLFGLLLAVRRSGRSLSLMLPLIRGLSKRLG

SEQ ID NO: 98 - protein, 32 aa, Artificial Sequence
  synthetic construct
MRLFGLLLAVRRSGRSLSLMLTPIRGLSKRLG

SEQ ID NO: 99 - protein, 32 aa, Artificial Sequence
  synthetic construct
MRLFGLLLAVRRSGRSLSLMLTLPRGLSKRLG

SEQ ID NO: 100 - protein, 32 aa, Artificial Sequence
  synthetic construct
MRLFGLLLAVRRSGRSLSLMLTLIPGLSKRLG

SEQ ID NO: 101 - protein, 32 aa, Artificial Sequence
  synthetic construct
MRLFGLLLAVRRSGRSLSLMLTLIRPLSKRLG

SEQ ID NO: 102 - protein, 32 aa, Artificial Sequence
  synthetic construct
MRLFGLLLAVRRSGRSLSLMLTLIRGPSKRLG

SEQ ID NO: 103 - protein, 32 aa, Artificial Sequence
  synthetic construct
MRLFGLLLAVRRSGRSLSLMLTLIRGLPKRLG

SEQ ID NO: 104 - protein, 32 aa, Artificial Sequence
  synthetic construct
MRLFGLLLAVRRSGRSLSLMLTLIRGLSPRLG

SEQ ID NO: 105 - protein, 32 aa, Artificial Sequence
  synthetic construct
MRLFGLLLAVRRSGRSLSLMLTLIRGLSKPLG

SEQ ID NO: 106 - protein, 32 aa, Artificial Sequence
  synthetic construct
MRLFGLLLAVRRSGRSLSLMLTLIRGLSKRPG

SEQ ID NO: 107 - protein, 32 aa, Artificial Sequence
  synthetic construct
MRLFGLLLAVRRSGRSLSLMLTLIRGLSKRLP

SEQ ID NO: 108 - protein, 32 aa, Artificial Sequence
  synthetic construct
MRLAALLLAARRSGRSLSLMLTLIRGLSKRLG

SEQ ID NO: 109 - protein, 32 aa, Artificial Sequence
  synthetic construct
MRLFALLLAARRSGRSLSLMLTLIRGLSKRLG

SEQ ID NO: 110 - protein, 32 aa, Artificial Sequence
  synthetic construct
MRLAGLLLAARRSGRSLSLMLTLIRGLSKRLG

SEQ ID NO: 111 - protein, 32 aa, Artificial Sequence
  synthetic construct
MRLAALLLAVRRSGRSLSLMLTLIRGLSKRLG

SEQ ID NO: 112 - protein, 32 aa, Artificial Sequence
  synthetic construct
MRLFGLLLAVRRSGRSPSPMPTPIPGPSKPPG

SEQ ID NO: 113 - protein, 32 aa, Artificial Sequence
  synthetic construct
MRLFGLLLAVRRSGRSPSLMPTPIPGPSKPPG

SEQ ID NO: 114 - protein, 32 aa, Artificial Sequence
  synthetic construct
MRLFGLLLAVRRSGRSPSLMPTLIPGPSKPPG

SEQ ID NO: 115 - protein, 32 aa, Artificial Sequence
  synthetic construct
MRLFGLLLAVRRSGRSPSLMPTLIPGLSKPPG

SEQ ID NO: 116 - protein, 32 aa, Artificial Sequence
  synthetic construct
MRLFGLLLAVRRSGRSPSLMPTLIPGLSKPLG

SEQ ID NO: 117 - protein, 32 aa, Artificial Sequence
  synthetic construct
MRLFGLLLAVRRSGRSLSLMPTLIPGLSKPLG

SEQ ID NO: 118 - protein, 32 aa, Artificial Sequence
  synthetic construct
MRLFGLLLAVRRSGRSLSLMPTLIPGLSKRLG

SEQ ID NO: 119 - protein, 32 aa, Artificial Sequence; identical to SEQ ID NO: 100
  synthetic construct

SEQ ID NO: 120 - protein, 32 aa, Artificial Sequence
  synthetic construct
MRLAALLLAARRSGRSPSPMPTPIPGPSKPPG

SEQ ID NO: 121 - protein, 32 aa, Artificial Sequence
  synthetic construct
MRLAALLLAARRSGRSPSLMPTPIPGPSKPPG

SEQ ID NO: 122 - protein, 32 aa, Artificial Sequence
  synthetic construct
MRLAALLLAARRSGRSPSLMPTLIPGPSKPPG

SEQ ID NO: 123 - protein, 32 aa, Artificial Sequence
  synthetic construct
MRLAALLLAARRSGRSPSLMPTLIPGLSKPPG

SEQ ID NO: 124 - protein, 32 aa, Artificial Sequence
  synthetic construct
MRLAALLLAARRSGRSPSLMPTLIPGLSKPLG

SEQ ID NO: 125 - protein, 32 aa, Artificial Sequence
  synthetic construct
MRLAALLLAARRSGRSLSLMPTLIPGLSKPLG

SEQ ID NO: 126 - protein, 32 aa, Artificial Sequence
  synthetic construct
MRLAALLLAARRSGRSLSLMPTLIPGLSKRLG

SEQ ID NO: 127 - protein, 32 aa, Artificial Sequence
  synthetic construct
MRLAALLLAARRSGRSLSLMLTLIPGLSKRLG

SEQ ID NO: 128 - protein, 32 aa, Artificial Sequence
  synthetic construct
MRLFALLLAARRSGRSPSPMPTPIPGPSKPPG

SEQ ID NO: 129 - protein, 32 aa, Artificial Sequence
  synthetic construct
MRLFALLLAARRSGRSPSLMPTPIPGPSKPPG

SEQ ID NO: 130 - protein, 32 aa, Artificial Sequence
  synthetic construct
MRLFALLLAARRSGRSPSLMPTLIPGPSKPPG

SEQ ID NO: 131 - protein, 32 aa, Artificial Sequence
  synthetic construct
MRLFALLLAARRSGRSPSLMPTLIPGLSKPPG

SEQ ID NO: 132 - protein, 32 aa, Artificial Sequence
  synthetic construct
MRLFALLLAARRSGRSPSLMPTLIPGLSKPLG

SEQ ID NO: 133 - protein, 32 aa, Artificial Sequence
  synthetic construct
MRLFALLLAARRSGRSLSLMPTLIPGLSKPLG

SEQ ID NO: 134 - protein, 32 aa, Artificial Sequence
  synthetic construct
MRLFALLLAARRSGRSLSLMPTLIPGLSKRLG

SEQ ID NO: 135 - protein, 32 aa, Artificial Sequence
  synthetic construct
MRLFALLLAARRSGRSLSLMLTLIPGLSKRLG

SEQ ID NO: 136 - protein, 32 aa, Artificial Sequence
  synthetic construct
MRLAGLLLAARRSGRSPSPMPTPIPGPSKPPG

SEQ ID NO: 137 - protein, 32 aa, Artificial Sequence
  synthetic construct
MRLAGLLLAARRSGRSPSLMPTPIPGPSKPPG

SEQ ID NO: 138 - protein, 32 aa, Artificial Sequence
  synthetic construct
MRLAGLLLAARRSGRSPSLMPTLIPGPSKPPG

SEQ ID NO: 139 - protein, 32 aa, Artificial Sequence
  synthetic construct
MRLAGLLLAARRSGRSPSLMPTLIPGLSKPPG

SEQ ID NO: 140 - protein, 32 aa, Artificial Sequence
  synthetic construct
MRLAGLLLAARRSGRSPSLMPTLIPGLSKPLG

SEQ ID NO: 141 - protein, 32 aa, Artificial Sequence
  synthetic construct
MRLAGLLLAARRSGRSLSLMPTLIPGLSKPLG

SEQ ID NO: 142 - protein, 32 aa, Artificial Sequence
  synthetic construct
MRLAGLLLAARRSGRSLSLMPTLIPGLSKRLG

SEQ ID NO: 143 - protein, 32 aa, Artificial Sequence
  synthetic construct
MRLAGLLLAARRSGRSLSLMLTLIPGLSKRLG

SEQ ID NO: 144 - protein, 32 aa, Artificial Sequence
  synthetic construct
MRLAALLLAVRRSGRSPSPMPTPIPGPSKPPG

SEQ ID NO: 145 - protein, 32 aa, Artificial Sequence
  synthetic construct
MRLAALLLAVRRSGRSPSLMPTPIPGPSKPPG

SEQ ID NO: 146 - protein, 32 aa, Artificial Sequence
  synthetic construct
MRLAALLLAVRRSGRSPSLMPTLIPGPSKPPG

SEQ ID NO: 147 - protein, 32 aa, Artificial Sequence
  synthetic construct
MRLAALLLAVRRSGRSPSLMPTLIPGLSKPPG

SEQ ID NO: 148 - protein, 32 aa, Artificial Sequence
  synthetic construct
MRLAALLLAVRRSGRSPSLMPTLIPGLSKPLG

SEQ ID NO: 149 - protein, 32 aa, Artificial Sequence
  synthetic construct
MRLAALLLAVRRSGRSLSLMPTLIPGLSKPLG

SEQ ID NO: 150 - protein, 32 aa, Artificial Sequence
  synthetic construct
MRLAALLLAVRRSGRSLSLMPTLIPGLSKRLG

SEQ ID NO: 151 - protein, 32 aa, Artificial Sequence
  synthetic construct
MRLAALLLAVRRSGRSLSLMLTLIPGLSKRLG

SEQ ID NO: 152 - protein, 32 aa, Artificial Sequence
  synthetic construct
MPLFGLLLPVPPSGRSLSLMLTLIRGLSKRLG

SEQ ID NO: 153 - protein, 32 aa, Artificial Sequence
  synthetic construct
MPLFGLLLPVPRSGRSLSLMLTLIRGLSKRLG

SEQ ID NO: 154 - protein, 32 aa, Artificial Sequence
  synthetic construct
MPLFGLLLPVRRSGRSLSLMLTLIRGLSKRLG

SEQ ID NO: 155 - protein, 32 aa, Artificial Sequence
  synthetic construct
MRLFGLLLAVRRSGRSLSLMLALIRALSKRLA

SEQ ID NO: 156 - protein, 32 aa, Artificial Sequence
  synthetic construct
MRLFGLLLAVRRSGRSLSLMLTLIRALSKRLA

SEQ ID NO: 157 - protein, 32 aa, Artificial Sequence
  synthetic construct
MRLFGLLLAVRRSGRSLSLMLALIRALSKRLG

SEQ ID NO: 158 - protein, 32 aa, Artificial Sequence
  synthetic construct
MRLFGLLLAVRRSGRSLSLMLALIRGLSKRLA

SEQ ID NO: 159 - protein, 32 aa, Artificial Sequence
  synthetic construct
MPLFGLLLPVPPSGRSLSLMLALIRALSKRLA

SEQ ID NO: 160 - protein, 32 aa, Artificial Sequence
  synthetic construct
MPLFGLLLPVPPSGRSLSLMLTLIRALSKRLA

SEQ ID NO: 161 - protein, 32 aa, Artificial Sequence
  synthetic construct
MPLFGLLLPVPPSGRSLSLMLALIRALSKRLG

SEQ ID NO: 162 - protein, 32 aa, Artificial Sequence
  synthetic construct
MPLFGLLLPVPPSGRSLSLMLALIRGLSKRLA

SEQ ID NO: 163 - protein, 32 aa, Artificial Sequence
  synthetic construct
MPLFGLLLPVPRSGRSLSLMLALIRALSKRLA

SEQ ID NO: 164 - protein, 32 aa, Artificial Sequence
  synthetic construct
MPLFGLLLPVPRSGRSLSLMLTLIRALSKRLA

SEQ ID NO: 165 - protein, 32 aa, Artificial Sequence
  synthetic construct
MPLFGLLLPVPRSGRSLSLMLALIRALSKRLG

SEQ ID NO: 166 - protein, 32 aa, Artificial Sequence
  synthetic construct
MPLFGLLLPVPRSGRSLSLMLALIRGLSKRLA

SEQ ID NO: 167 - protein, 32 aa, Artificial Sequence
  synthetic construct
MPLFGLLLPVRRSGRSLSLMLALIRALSKRLA

SEQ ID NO: 168 - protein, 32 aa, Artificial Sequence
  synthetic construct
MPLFGLLLPVRRSGRSLSLMLTLIRALSKRLA

SEQ ID NO: 169 - protein, 32 aa, Artificial Sequence
  synthetic construct
MPLFGLLLPVRRSGRSLSLMLALIRALSKRLG

SEQ ID NO: 170 - protein, 32 aa, Artificial Sequence
  synthetic construct
MPLFGLLLPVRRSGRSLSLMLALIRGLSKRLA

SEQ ID NO: 171 - protein, 32 aa, Artificial Sequence
  synthetic construct
MPLFGLLLPVPPSGRSPSPMPTPIPGPSKPPG

SEQ ID NO: 172 - protein, 32 aa, Artificial Sequence
  synthetic construct
MPLFGLLLPVPPSGRSPSLMPTPIPGPSKPPG

SEQ ID NO: 173 - protein, 32 aa, Artificial Sequence
  synthetic construct
MPLFGLLLPVPPSGRSPSLMPTLIPGPSKPPG

SEQ ID NO: 174 - protein, 32 aa, Artificial Sequence
  synthetic construct
MPLFGLLLPVPPSGRSPSLMPTLIPGLSKPPG

SEQ ID NO: 175 - protein, 32 aa, Artificial Sequence
  synthetic construct
MPLFGLLLPVPPSGRSPSLMPTLIPGLSKPLG

SEQ ID NO: 176 - protein, 32 aa, Artificial Sequence
  synthetic construct
MPLFGLLLPVPPSGRSLSLMPTLIPGLSKPLG

SEQ ID NO: 177 - protein, 32 aa, Artificial Sequence
  synthetic construct
MPLFGLLLPVPPSGRSLSLMPTLIPGLSKRLG

SEQ ID NO: 178 - protein, 32 aa, Artificial Sequence
  synthetic construct
MPLFGLLLPVPPSGRSLSLMLTLIPGLSKRLG

SEQ ID NO: 179 - protein, 32 aa, Artificial Sequence
  synthetic construct
MPLFGLLLPVPRSGRSPSPMPTPIPGPSKPPG

SEQ ID NO: 180 - protein, 32 aa, Artificial Sequence
  synthetic construct
MPLFGLLLPVPRSGRSPSLMPTPIPGPSKPPG

SEQ ID NO: 181 - protein, 32 aa, Artificial Sequence
  synthetic construct
MPLFGLLLPVPRSGRSPSLMPTLIPGPSKPPG

SEQ ID NO: 182 - protein, 32 aa, Artificial Sequence
  synthetic construct
MPLFGLLLPVPRSGRSPSLMPTLIPGLSKPPG

SEQ ID NO: 183 - protein, 32 aa, Artificial Sequence
  synthetic construct
MPLFGLLLPVPRSGRSPSLMPTLIPGLSKPLG

SEQ ID NO: 184 - protein, 32 aa, Artificial Sequence
  synthetic construct
MPLFGLLLPVPRSGRSLSLMPTLIPGLSKPLG

SEQ ID NO: 185 - protein, 32 aa, Artificial Sequence
  synthetic construct
MPLFGLLLPVPRSGRSLSLMPTLIPGLSKRLG

SEQ ID NO: 186 - protein, 32 aa, Artificial Sequence
  synthetic construct
MPLFGLLLPVPRSGRSLSLMLTLIPGLSKRLG

SEQ ID NO: 187 - protein, 32 aa, Artificial Sequence
  synthetic construct
MPLFGLLLPVRRSGRSPSPMPTPIPGPSKPPG

SEQ ID NO: 188 - protein, 32 aa, Artificial Sequence
  synthetic construct
MPLFGLLLPVRRSGRSPSLMPTPIPGPSKPPG

SEQ ID NO: 189 - protein, 32 aa, Artificial Sequence
  synthetic construct
MPLFGLLLPVRRSGRSPSLMPTLIPGPSKPPG

SEQ ID NO: 190 - protein, 32 aa, Artificial Sequence
  synthetic construct
MPLFGLLLPVRRSGRSPSLMPTLIPGLSKPPG

SEQ ID NO: 191 - protein, 32 aa, Artificial Sequence
  synthetic construct
MPLFGLLLPVRRSGRSPSLMPTLIPGLSKPLG

SEQ ID NO: 192 - protein, 32 aa, Artificial Sequence
  synthetic construct
MPLFGLLLPVRRSGRSLSLMPTLIPGLSKPLG

SEQ ID NO: 193 - protein, 32 aa, Artificial Sequence
  synthetic construct
MPLFGLLLPVRRSGRSLSLMPTLIPGLSKRLG

SEQ ID NO: 194 - protein, 32 aa, Artificial Sequence
  synthetic construct
MPLFGLLLPVRRSGRSLSLMLTLIPGLSKRLG

SEQ ID NO: 195 - protein, 32 aa, Artificial Sequence
  synthetic construct
MRLAALLLAARRSGRSLSLMLALIRALSKRLA

SEQ ID NO: 196 - protein, 32 aa, Artificial Sequence
  synthetic construct
MRLAALLLAARRSGRSLSLMLTLIRALSKRLA

SEQ ID NO: 197 - protein, 32 aa, Artificial Sequence
  synthetic construct
MRLAALLLAARRSGRSLSLMLALIRALSKRLG

SEQ ID NO: 198 - protein, 32 aa, Artificial Sequence
  synthetic construct
MRLAALLLAARRSGRSLSLMLALIRGLSKRLA

SEQ ID NO: 199 - protein, 32 aa, Artificial Sequence
  synthetic construct
MRLFALLLAARRSGRSLSLMLALIRALSKRLA

SEQ ID NO: 200 - protein, 32 aa, Artificial Sequence
  synthetic construct
MRLFALLLAARRSGRSLSLMLTLIRALSKRLA

SEQ ID NO: 201 - protein, 32 aa, Artificial Sequence
  synthetic construct
MRLFALLLAARRSGRSLSLMLALIRALSKRLG

SEQ ID NO: 202 - protein, 32 aa, Artificial Sequence
  synthetic construct
MRLFALLLAARRSGRSLSLMLALIRGLSKRLA

SEQ ID NO: 203 - protein, 32 aa, Artificial Sequence
  synthetic construct
MRLAGLLLAARRSGRSLSLMLALIRALSKRLA

SEQ ID NO: 204 - protein, 32 aa, Artificial Sequence
  synthetic construct
MRLAGLLLAARRSGRSLSLMLTLIRALSKRLA

SEQ ID NO: 205 - protein, 32 aa, Artificial Sequence
  synthetic construct
MRLAGLLLAARRSGRSLSLMLALIRALSKRLG

SEQ ID NO: 206 - protein, 32 aa, Artificial Sequence
  synthetic construct
MRLAGLLLAARRSGRSLSLMLALIRGLSKRLA

SEQ ID NO: 207 - protein, 32 aa, Artificial Sequence
  synthetic construct
MRLAALLLAVRRSGRSLSLMLALIRALSKRLA

SEQ ID NO: 208 - protein, 32 aa, Artificial Sequence
  synthetic construct
MRLAALLLAVRRSGRSLSLMLTLIRALSKRLA

SEQ ID NO: 209 - protein, 32 aa, Artificial Sequence
  synthetic construct
MRLAALLLAVRRSGRSLSLMLALIRALSKRLG

SEQ ID NO: 210 - protein, 32 aa, Artificial Sequence
  synthetic construct
MRLAALLLAVRRSGRSLSLMLALIRGLSKRLA

SEQ ID NO: 211 - protein, 32 aa, Artificial Sequence
  synthetic construct
MRLFGLLLAVRRSGRSLSLMLDLIRGLSKRLG

SEQ ID NO: 212 - protein, 32 aa, Artificial Sequence
  synthetic construct
MRLFGLLLAVRRSGRSLSLMLRLIRGLSKRLG

SEQ ID NO: 213 - protein, 32 aa, Artificial Sequence
  synthetic construct
MRLFGLLLAVRRSGRSLSLMLWLIRGLSKRLG

SEQ ID NO: 214 - protein, 32 aa, Artificial Sequence
  synthetic construct
MRLFGLLLAVRRSGRSLSLMLKLIRGLSKRLG

SEQ ID NO: 215 - protein, 32 aa, Homo sapiens; identical to SEQ ID NO: 9